European Patent Specification EP 3 446 126 B1, published June 12, 2024. Title: A NEW BIOMARKER EXPRESSED IN PANCREATIC BETA CELLS USEFUL IN IMAGING OR TARGETING BETA CELLS. Applicant: Vrije Universiteit Brussel Université Libre de Bruxelles. The sequence listing filed with the application follows.

SEQUENCE LISTING (11 sequences)

SEQ ID NO: 1 - protein, 801 aa, Homo Sapiens
MKEKAMIKTAKMQGNVMELVGSNPPQRNWKGIAIALLVILVICSLIVTSVILLTPAEDNSLSQKKKVTVEDLFSEDFKIHDPEAKWISDTEFIYREQKGTVRLWNVETNTSTVLIEGKKIESLRAIRYEISPDREYALFSYNVEPIYQHSYTGYYVLSKIPHGDPQSLDPPEVSNAKLQYAGWGPKGQQLIFIFENNIYYCAHVGKQAIRVVSTGKEGVIYNGLSDWLYEEEILKTHIAHWWSPDGTRLAYAAINDSRVPIMELPTYTGSIYPTVKPYHYPKAGSENPSISLHVIGLNGPTHDLEMMPPDDPRMREYYITMVKWATSTKVAVTWLNRAQNVSILTLCDATTGVCTKKHEDESEAWLHRQNEEPVFSKDGRKFFFIRAIPQGGRGKFYHITVSSSQPNSSNDNIQSITSGDWDVTKILAYDEKGNKIYFLSTEDLPRRRQLYSANTVGNFNRQCLSCDLVENCTYFSASFSHSMDFFLLKCEGPGVPMVTVHNTTDKKKMFDLETNEHVKKAINDRQMPKVEYRDIEIDDYNLPMQILKPATFTDTTHYPLLLVVDGTPGSQSVAEKFEVSWETVMVSSHGAVVVKCDGRGSGFQGTKLLHEVRRRLGLLEEKDQMEAVRTMLKEQYIDRTRVAVFGKDYGGYLSTYILPAKGENQGQTFTCGSALSPITDFKLYASAFSERYLGLHGLDNRAYEMTKVAHRVSALEEQQFLIIHPTADEKIHFQHTAELITQLIRGKANYSLQIYPDESHYFTSSSLKQHLYRSIINFFVECFRIQDKLLTVTAKEDEEED

SEQ ID NO: 2 - protein, 801 aa, Homo Sapiens
MKEKAMIKTAKMQGNVMELVGSNPPQRNWKGIAIALLVILVICSLIVTSVILLTPAEDTSLSQKKKVTVEDLFSEDFKIHDPEAKWISNKEFIYRERKGSVILRNVETNNSTVLIEGKKIESLRAIRYEISPDKEYVLFSYNVEPVYQHSHTGYYVLSKIPHGDPQSLDPPEVSNAKLQYAGWGPKGQQLIFIFENNIYYCAHVGKQAIRVVSTGKEGVIYNGLSDWLYEEEILKSHIAHWWSPDGTRLAYATINDSRVPLMELPTYTGSVYPTVKPYHYPKAGSENPSISLHVIGLNGPTHDLEMMPPDDPRMREYYITMVKWATSTKVAVTWLNRAQNVSILTLCDATTGVCTKKHEDESEAWLHRQNEEPVFSKDGRKFFFVRAIPQGGRGKFYHITVSSSQPNSSNDNIQSITSGDWDVTKILSYDEKRNKIYFLSTEDLPRRRHLYSANTVDDFNRQCLSCDLVENCTYVSASFSHNMDFFLLKCEGPGVPTVTVHNTTDKRRMFDLEANEEVQKAINDRQMPKIEYRKIEVEDYSLPMQILKPATFTDTAHYPLLLVVDGTPGSQSVTERFEVTWETVLVSSHGAVVVKCDGRGSGFQGTKLLQEVRRRLGFLEEKDQMEAVRTMLKEQYIDKTRVAVFGKDYGGYLSTYILPAKGENQGQTFTCGSALSPITDFKLYASAFSERYLGLHGLDNRAYEMTKLAHRVSALEDQQFLIIHATADEKIHFQHTAELITQLIKGKANYSLQIYPDESHYFHSVALKQHLSRSIIGFFVECFRVQDKLPTATAKEEEEED

SEQ ID NO: 3 - protein, 749 aa, Homo Sapiens
LTPAEDNSLSQKKKVTVEDLFSEDFKIHDPEAKWISDTEFIYREQKGTVRLWNVETNTSTVLIEGKKIESLRAIRYEISPDREYALFSYNVEPIYQHSYTGYYVLSKIPHGDPQSLDPPEVSNAKLQYAGWGPKGQQLIFIFENNIYYCAHVGKQAIRVVSTGKEGVIYNGLSDWLYEEEILKTHIAHWWSPDGTRLAYAAINDSRVPIMELPTYTGSIYPTVKPYHYPKAGSENPSISLHVIGLNGPTHDLEMMPPDDPRMREYYITMVKWATSTKVAVTWLNRAQNVSILTLCDATTGVCTKKHEDESEAWLHRQNEEPVFSKDGRKFFFIRAIPQGGRGKFYHITVSSSQPNSSNDNIQSITSGDWDVTKILAYDEKGNKIYFLSTEDLPRRRQLYSANTVGNFNRQCLSCDLVENCTYFSASFSHSMDFFLLKCEGPGVPMVTVHNTTDKKKMFDLETNEHVKKAINDRQMPKVEYRDIEIDDYNLPMQILKPATFTDTTHYPLLLVVDGTPGSQSVAEKFEVSWETVMVSSHGAVVVKCDGRGSGFQGTKLLHEVRRRLGLLEEKDQMEAVRTMLKEQYIDRTRVAVFGKDYGGYLSTYILPAKGENQGQTFTCGSALSPITDFKLYASAFSERYLGLHGLDNRAYEMTKVAHRVSALEEQQFLIIHPTADEKIHFQHTAELITQLIRGKANYSLQIYPDESHYFTSSSLKQHLYRSIINFFVECFRIQDKLLTVTAKEDEEED

SEQ ID NO: 4 - DNA, 23 bp, Artificial
  Primer
acagtgagactgtggaatgttga

SEQ ID NO: 5 - DNA, 23 bp, Artificial
  Primer
gaggatccccatgaggaattttg

SEQ ID NO: 6 - DNA, 25 bp, Artificial
  Primer
gcctggagaaacctgccaagtatga

SEQ ID NO: 7 - DNA, 22 bp, Artificial
  Primer
aacctggtcctcagtgtagccc

SEQ ID NO: 8 - protein, 119 aa, Artificial
  Nanobody
QVQLQESGGGLVQPGGSLRLSCAASGFTFSSNYMTWVRQAPGKGPEWVSGINPDGSSTYYADSVKGRFTISRDNAKNTLYLQMNSLKSEDTALYKCATGAAPRIPTTLRGQGTQVTVSS

SEQ ID NO: 9 - protein, 8 aa, Artificial
  CDR region of nanobody
GFTFSSNY

SEQ ID NO: 10 - protein, 8 aa, Artificial
  CDR region of nanobody
INPDGSST

SEQ ID NO: 11 - protein, 12 aa, Artificial
  CDR region of nanobody
ATGAAPRIPTTL